European Patent Application EP 4 265 274 A1, published October 25, 2023. Title: B7-H3 TARGETING ANTIBODY-DRUG CONJUGATE, AND PREPARATION METHOD THEREFOR AND USE THEREOF. Applicant: Shanghai Fudan-Zhangjiang Bio-Pharmaceutical Co.,Ltd. The sequence listing filed with the application follows.

SEQUENCE LISTING (2 sequences)

SEQ ID NO: 1 - protein, 215 aa, Homo sapiens
DIQMTQSPSSLSASVGDRVTITCRASESIYSYLAWYQQKPGKAPKLLVYNTKTLPEGVPSRFSGSGSGTDFTLTISSLQPEDFATYYCQHHYGTPPWTFGQGTRLEIKRTVAAPSVFIFPPSDEQLKSGTASVVCLLNNFYPREAKVQWKVDNALQSGNSQESVTEQDSKDSTYSLSSTLTLSKADYEKHKVYACEVTHQGLSSPVTKSFNRGEC

SEQ ID NO: 2 - protein, 447 aa, Homo sapiens
EVQLVESGGGLVKPGGSLRLSCAASGFTFSSYGMSWVRQAPGKGLEWVATINSGGSNTYYPDSLKGRFTISRDNAKNSLYLQMNSLRAEDTAVYYCARHDGGAMDYWGQGTTVTVSSASTKGPSVFPLAPSSKSTSGGTAALGCLVKDYFPEPVTVSWNSGALTSGVHTFPAVLQSSGLYSLSSVVTVPSSSLGTQTYICNVNHKPSNTKVDKRVEPKSCDKTHTCPPCPAPELLGGPSVFLFPPKPKDTLMISRTPEVTCVVVDVSHEDPEVKFNWYVDGVEVHNAKTKPREEQYNSTYRVVSVLTVLHQDWLNGKEYKCKVSNKALPAPIEKTISKAKGQPREPQVYTLPPSREEMTKNQVSLTCLVKGFYPSDIAVEWESNGQPENNYKTTPPVLDSDGSFFLYSKLTVDKSRWQQGNVFSCSVMHEALHNHYTQKSLSLSPGK